European Patent Application EP 4 725 560 A2, published April 15, 2026. Title: Anti-B7H3 antibodies for the preparation of antibody drug conjugates (ADCs) of KSP inhibitors. Applicant: BAYER AG. Application EP. The sequence listing filed with the application follows.

SEQUENCE LISTING (70 sequences)

SEQ ID NO: 1 - protein, 117 aa, unidentified
EVQLLESGGGLVQPGGSLRLSCAASGFTFRSYAMSWVRQAPGKGLEWVSSVSGSGGSALYADSVKGRFTISRDNSKNTLYLQMNSLRAEDTAVYYCTRLTGTSFDYWGQGTLVTVSS

SEQ ID NO: 2 - protein, 5 aa, unidentified
SYAMS

SEQ ID NO: 3 - protein, 17 aa, unidentified
SVSGSGGSALYADSVKG

SEQ ID NO: 4 - protein, 8 aa, unidentified
LTGTSFDY

SEQ ID NO: 5 - protein, 109 aa, unidentified
QSVLTQPPSASGTPGQRVTISCSGSSSNIGSNPVNWYQQLPGTAPKLLIYGNSNRPSGVPDRFSGSKSGTSASLAISGLRSEDEADYYCQSFDSSLKKVFGGGTKLTVL

SEQ ID NO: 6 - protein, 13 aa, unidentified
SGSSSNIGSNPVN

SEQ ID NO: 7 - protein, 7 aa, unidentified
GNSNRPS

SEQ ID NO: 8 - protein, 10 aa, unidentified
QSFDSSLKKV

SEQ ID NO: 9 - protein, 446 aa, unidentified
EVQLLESGGGLVQPGGSLRLSCAASGFTFRSYAMSWVRQAPGKGLEWVSSVSGSGGSALYADSVKGRFTISRDNSKNTLYLQMNSLRAEDTAVYYCTRLTGTSFDYWGQGTLVTVSSASTKGPSVFPLAPSSKSTSGGTAALGCLVKDYFPEPVTVSWNSGALTSGVHTFPAVLQSSGLYSLSSVVTVPSSSLGTQTYICNVNHKPSNTKVDKKVEPKSCDKTHTCPPCPAPELLGGPSVFLFPPKPKDTLMISRTPEVTCVVVDVSHEDPEVKFNWYVDGVEVHNAKTKPREEQYNSTYRVVSVLTVLHQDWLNGKEYKCKVSNKALPAPIEKTISKAKGQPREPQVYTLPPSRDELTKNQVSLTCLVKGFYPSDIAVEWESNGQPENNYKTTPPVLDSDGSFFLYSKLTVDKSRWQQGNVFSCSVMHEALHNHYTQKSLSLSPG

SEQ ID NO: 10 - protein, 215 aa, unidentified
QSVLTQPPSASGTPGQRVTISCSGSSSNIGSNPVNWYQQLPGTAPKLLIYGNSNRPSGVPDRFSGSKSGTSASLAISGLRSEDEADYYCQSFDSSLKKVFGGGTKLTVLGQPKAAPSVTLFPPSSEELQANKATLVCLISDFYPGAVTVAWKADSSPVKAGVETTTPSKQSNNKYAASSYLSLTPEQWKSHRSYSCQVTHEGSTVEKTVAPTECS

SEQ ID NO: 11 - protein, 125 aa, unidentified
EVQLLESGGGLVQPGGSLRLSCAASGFTFRDFYMNWIRQAPGKGLEWVSSISASGKYTYYADSVKGRFTISRDNSKNTLYLQMNSLRAEDTAVYYCAREWGYCTNDVCRNWFDPWGQGTLVTVSS

SEQ ID NO: 12 - protein, 5 aa, unidentified
DFYMN

SEQ ID NO: 13 - protein, 17 aa, unidentified
SISASGKYTYYADSVKG

SEQ ID NO: 14 - protein, 16 aa, unidentified
EWGYCTNDVCRNWFDP

SEQ ID NO: 15 - protein, 110 aa, unidentified
QSVLTQPPSASGTPGQRVTISCSGGYSNVGGNNVNWYQQLPGTAPKLLIYGNSNRPSGVPDRFSGSKSGTSASLAISGLRSEDEADYYCQSYDSSLSGSVFGGGTKLTVL

SEQ ID NO: 16 - protein, 13 aa, unidentified
SGGYSNVGGNNVN

SEQ ID NO: 17 - protein, 7 aa, unidentified
GNSNRPS

SEQ ID NO: 18 - protein, 11 aa, unidentified
QSYDSSLSGSV

SEQ ID NO: 19 - protein, 454 aa, unidentified
EVQLLESGGGLVQPGGSLRLSCAASGFTFRDFYMNWIRQAPGKGLEWVSSISASGKYTYYADSVKGRFTISRDNSKNTLYLQMNSLRAEDTAVYYCAREWGYCTNDVCRNWFDPWGQGTLVTVSSASTKGPSVFPLAPSSKSTSGGTAALGCLVKDYFPEPVTVSWNSGALTSGVHTFPAVLQSSGLYSLSSVVTVPSSSLGTQTYICNVNHKPSNTKVDKKVEPKSCDKTHTCPPCPAPELLGGPSVFLFPPKPKDTLMISRTPEVTCVVVDVSHEDPEVKFNWYVDGVEVHNAKTKPREEQYNSTYRVVSVLTVLHQDWLNGKEYKCKVSNKALPAPIEKTISKAKGQPREPQVYTLPPSRDELTKNQVSLTCLVKGFYPSDIAVEWESNGQPENNYKTTPPVLDSDGSFFLYSKLTVDKSRWQQGNVFSCSVMHEALHNHYTQKSLSLSPG

SEQ ID NO: 20 - protein, 216 aa, unidentified
QSVLTQPPSASGTPGQRVTISCSGGYSNVGGNNVNWYQQLPGTAPKLLIYGNSNRPSGVPDRFSGSKSGTSASLAISGLRSEDEADYYCQSYDSSLSGSVFGGGTKLTVLGQPKAAPSVTLFPPSSEELQANKATLVCLISDFYPGAVTVAWKADSSPVKAGVETTTPSKQSNNKYAASSYLSLTPEQWKSHRSYSCQVTHEGSTVEKTVAPTECS

SEQ ID NO: 21 - protein, 118 aa, unidentified
EVQLLESGGGLVQPGGSLRLSCAASGFTFSSYGMHWVRQAPGKGLEWVSAISGSGGSTYYADSVKGRFTISRDNSKNTLYLQMNSLRAEDTAVYYCARGSNYLGMDVWGQGTLVTVSS

SEQ ID NO: 22 - protein, 5 aa, unidentified
SYGMH

SEQ ID NO: 23 - protein, 17 aa, unidentified
AISGSGGSTYYADSVKG

SEQ ID NO: 24 - protein, 9 aa, unidentified
GSNYLGMDV

SEQ ID NO: 25 - protein, 107 aa, unidentified
QSVLTQPPSASGTPGQRVTISCSGSSSNIGRNIVNWYQQLPGTAPKLLIYRSNQRPSGVPDRFSGSKSGTSASLAISGLRSEDEADYYCQTWGTGWVFGGGTKLTVL

SEQ ID NO: 26 - protein, 13 aa, unidentified
SGSSSNIGRNIVN

SEQ ID NO: 27 - protein, 7 aa, unidentified
RSNQRPS

SEQ ID NO: 28 - protein, 8 aa, unidentified
QTWGTGWV

SEQ ID NO: 29 - protein, 447 aa, unidentified
EVQLLESGGGLVQPGGSLRLSCAASGFTFSSYGMHWVRQAPGKGLEWVSAISGSGGSTYYADSVKGRFTISRDNSKNTLYLQMNSLRAEDTAVYYCARGSNYLGMDVWGQGTLVTVSSASTKGPSVFPLAPSSKSTSGGTAALGCLVKDYFPEPVTVSWNSGALTSGVHTFPAVLQSSGLYSLSSVVTVPSSSLGTQTYICNVNHKPSNTKVDKKVEPKSCDKTHTCPPCPAPELLGGPSVFLFPPKPKDTLMISRTPEVTCVVVDVSHEDPEVKFNWYVDGVEVHNAKTKPREEQYNSTYRVVSVLTVLHQDWLNGKEYKCKVSNKALPAPIEKTISKAKGQPREPQVYTLPPSRDELTKNQVSLTCLVKGFYPSDIAVEWESNGQPENNYKTTPPVLDSDGSFFLYSKLTVDKSRWQQGNVFSCSVMHEALHNHYTQKSLSLSPG

SEQ ID NO: 30 - protein, 213 aa, unidentified
QSVLTQPPSASGTPGQRVTISCSGSSSNIGRNIVNWYQQLPGTAPKLLIYRSNQRPSGVPDRFSGSKSGTSASLAISGLRSEDEADYYCQTWGTGWVFGGGTKLTVLGQPKAAPSVTLFPPSSEELQANKATLVCLISDFYPGAVTVAWKADSSPVKAGVETTTPSKQSNNKYAASSYLSLTPEQWKSHRSYSCQVTHEGSTVEKTVAPTECS

SEQ ID NO: 31 - protein, 118 aa, unidentified
EVQLLESGGGLVQPGGSLRLSCAASGFTFSTYGMHWVRQAPGKGLEWVSAISGSGGSTYYADSVKGRFTISRDNSKNTLYLQMNSLRAEDTAVYYCTRGYYYYGMDVWGQGTLVTVSS

SEQ ID NO: 32 - protein, 5 aa, unidentified
TYGMH

SEQ ID NO: 33 - protein, 17 aa, unidentified
AISGSGGSTYYADSVKG

SEQ ID NO: 34 - protein, 9 aa, unidentified
GYYYYGMDV

SEQ ID NO: 35 - protein, 110 aa, unidentified
QSVLTQPPSASGTPGQRVTISCSGGSSNIGSNPVNWYQQLPGTAPKLLIYGNSKRPSGVPDRFSGSKSGTSASLAISGLRSEDEADYYCQSYDSSLSGWVFGGGTKLTVL

SEQ ID NO: 36 - protein, 13 aa, unidentified
SGGSSNIGSNPVN

SEQ ID NO: 37 - protein, 7 aa, unidentified
GNSKRPS

SEQ ID NO: 38 - protein, 11 aa, unidentified
QSYDSSLSGWV

SEQ ID NO: 39 - protein, 447 aa, unidentified
EVQLLESGGGLVQPGGSLRLSCAASGFTFSTYGMHWVRQAPGKGLEWVSAISGSGGSTYYADSVKGRFTISRDNSKNTLYLQMNSLRAEDTAVYYCTRGYYYYGMDVWGQGTLVTVSSASTKGPSVFPLAPSSKSTSGGTAALGCLVKDYFPEPVTVSWNSGALTSGVHTFPAVLQSSGLYSLSSVVTVPSSSLGTQTYICNVNHKPSNTKVDKKVEPKSCDKTHTCPPCPAPELLGGPSVFLFPPKPKDTLMISRTPEVTCVVVDVSHEDPEVKFNWYVDGVEVHNAKTKPREEQYNSTYRVVSVLTVLHQDWLNGKEYKCKVSNKALPAPIEKTISKAKGQPREPQVYTLPPSRDELTKNQVSLTCLVKGFYPSDIAVEWESNGQPENNYKTTPPVLDSDGSFFLYSKLTVDKSRWQQGNVFSCSVMHEALHNHYTQKSLSLSPG

SEQ ID NO: 40 - protein, 216 aa, unidentified
QSVLTQPPSASGTPGQRVTISCSGGSSNIGSNPVNWYQQLPGTAPKLLIYGNSKRPSGVPDRFSGSKSGTSASLAISGLRSEDEADYYCQSYDSSLSGWVFGGGTKLTVLGQPKAAPSVTLFPPSSEELQANKATLVCLISDFYPGAVTVAWKADSSPVKAGVETTTPSKQSNNKYAASSYLSLTPEQWKSHRSYSCQVTHEGSTVEKTVAPTECS

SEQ ID NO: 41 - protein, 118 aa, unidentified
EVQLLESGGGLVQPGGSLRLSCAASGFTFSSYGMHWVRQVPGKGLEWVSAISGSGGTTYYADSVKGRFTISRDNSKNTLYLQMNSLRAEDTAVYYCARGGYHFLFDYWGQGTLVTVSS

SEQ ID NO: 42 - protein, 5 aa, unidentified
SYGMH

SEQ ID NO: 43 - protein, 17 aa, unidentified
AISGSGGTTYYADSVKG

SEQ ID NO: 44 - protein, 9 aa, unidentified
GGYHFLFDY

SEQ ID NO: 45 - protein, 110 aa, unidentified
QSVLTQPPSASGTPGQRVTISCSGSSSNIGSNTVNWYQQLPGTAPKLLIYRNDQRLLGVPDRFSGSKSGTSASLAISGLRSEDEADYYCQSYDSSLSGWVFGGGTKLTVL

SEQ ID NO: 46 - protein, 13 aa, unidentified
SGSSSNIGSNTVN

SEQ ID NO: 47 - protein, 7 aa, unidentified
RNDQRLL

SEQ ID NO: 48 - protein, 11 aa, unidentified
QSYDSSLSGWV

SEQ ID NO: 49 - protein, 447 aa, unidentified
EVQLLESGGGLVQPGGSLRLSCAASGFTFSSYGMHWVRQVPGKGLEWVSAISGSGGTTYYADSVKGRFTISRDNSKNTLYLQMNSLRAEDTAVYYCARGGYHFLFDYWGQGTLVTVSSASTKGPSVFPLAPSSKSTSGGTAALGCLVKDYFPEPVTVSWNSGALTSGVHTFPAVLQSSGLYSLSSVVTVPSSSLGTQTYICNVNHKPSNTKVDKKVEPKSCDKTHTCPPCPAPELLGGPSVFLFPPKPKDTLMISRTPEVTCVVVDVSHEDPEVKFNWYVDGVEVHNAKTKPREEQYNSTYRVVSVLTVLHQDWLNGKEYKCKVSNKALPAPIEKTISKAKGQPREPQVYTLPPSRDELTKNQVSLTCLVKGFYPSDIAVEWESNGQPENNYKTTPPVLDSDGSFFLYSKLTVDKSRWQQGNVFSCSVMHEALHNHYTQKSLSLSPG

SEQ ID NO: 50 - protein, 216 aa, unidentified
QSVLTQPPSASGTPGQRVTISCSGSSSNIGSNTVNWYQQLPGTAPKLLIYRNDQRLLGVPDRFSGSKSGTSASLAISGLRSEDEADYYCQSYDSSLSGWVFGGGTKLTVLGQPKAAPSVTLFPPSSEELQANKATLVCLISDFYPGAVTVAWKADSSPVKAGVETTTPSKQSNNKYAASSYLSLTPEQWKSHRSYSCQVTHEGSTVEKTVAPTECS

SEQ ID NO: 51 - protein, 296 aa, unidentified
EQAPGTAPCSRGSSWSADLDKCMDCASCRARPHSDFCLGCAAAPPAPFRLLWPIEGRMDPKSCDKTHTCPPCPAPELLGGPSVFLFPPKPKDTLMISRTPEVTCVVVDVSHEDPEVKFNWYVDGVEVHNAKTKPREEQYNSTYRVVSVLTVLHQDWLNGKEYKCKVSNKALPAPIEKTISKAKGQPREPQVYTLPPSREEMTKNQVSLTCLVKGFYPSDIAVEWESNGQPENNYKTTPPVLDSDGSFFLYSKLTVDKSRWQQGNVFSCSVMHEALHNHYTQKSLSLSPGKHHHHHH

SEQ ID NO: 52 - protein, 435 aa, unidentified
GALEVQVPEDPVVALVGTDATLCCSFSPEPGFSLAQLNLIWQLTDTKQLVHSFAEGQDQGSAYANRTALFPDLLAQGNASLRLQRVRVADEGSFTCFVSIRDFGSAAVSLQVAAPYSKPSMTLEPNKDLRPGDTVTITCSSYQGYPEAEVFWQDGQGVPLTGNVTTSQMANEQGLFDVHSILRVVLGANGTYSCLVRNPVLQQDAHSSVTITPQRSPTGAVEVQVPEDPVVALVGTDATLRCSFSPEPGFSLAQLNLIWQLTDTKQLVHSFTEGRDQGSAYANRTALFPDLLAQGNASLRLQRVRVADEGSFTCFVSIRDFGSAAVSLQVAAPYSKPSMTLEPNKDLRPGDTVTITCSSYRGYPEAEVFWQDGQGVPLTGNVTTSQMANEQGLFDVHSVLRVVLGANGTYSCLVRNPVLQQDAHGSVTITGQPMT

SEQ ID NO: 53 - protein, 216 aa, unidentified
VEVQVSEDPVVALVDTDATLRCSFSPEPGFSLAQLNLIWQLTDTKQLVHSFTEGRDQGSAYSNRTALFPDLLVQGNASLRLQRVRVTDEGSYTCFVSIQDFDSAAVSLQVAAPYSKPSMTLEPNKDLRPGNMVTITCSSYQGYPEAEVFWKDGQGVPLTGNVTTSQMANERGLFDVHSVLRVVLGANGTYSCLVRNPVLQQDAHGSVTITGQPLTF

SEQ ID NO: 54 - protein, 446 aa, unidentified
EVQLLESGGGLVQPGGSLRLSCAASGFTFRSYAMSWVRQAPGKGLEWVSSVSGSGGSALYADSVKGRFTISRDNSKNTLYLQMNSLRAEDTAVYYCTRLTGTSFDYWGQGTLVTVSSASTKGPSVFPLAPSSKSTSGGTAALGCLVKDYFPEPVTVSWNSGALTSGVHTFPAVLQSSGLYSLSSVVTVPSSSLGTQTYICNVNHKPSNTKVDKKVEPKSCDKTHTCPPCPAPELLGGPSVFLFPPKPKDTLMISRTPEVTCVVVDVSHEDPEVKFNWYVDGVEVHNAKTKPREEQYASTYRVVSVLTVLHQDWLNGKEYKCKVSNKALPAPIEKTISKAKGQPREPQVYTLPPSRDELTKNQVSLTCLVKGFYPSDIAVEWESNGQPENNYKTTPPVLDSDGSFFLYSKLTVDKSRWQQGNVFSCSVMHEALHNHYTQKSLSLSPG

SEQ ID NO: 55 - protein, 117 aa, unidentified
EVQLLESGGGLVQPGGSLRLSCAASGFTFSSYAMSWVRQAPGKGLEWVSSISGSGGSTLYADSVKGRFTISRDNSKNTLYLQMNSLRAEDTAVYYCAKLTGTSFDYWGQGTLVTVSS

SEQ ID NO: 56 - protein, 17 aa, unidentified
SISGSGGSTLYADSVKG

SEQ ID NO: 57 - protein, 109 aa, unidentified
QSVLTQPPSASGTPGQRVTISCSGSSSNIGSNPVNWYQQLPGTAPKLLIYSNNQRPSGVPDRFSGSKSGTSASLAITGLQSEDEADYYCQSFDSSLKKVFGGGTKLTVL

SEQ ID NO: 58 - protein, 7 aa, unidentified
SNNQRPS

SEQ ID NO: 59 - protein, 446 aa, unidentified
EVQLLESGGGLVQPGGSLRLSCAASGFTFSSYAMSWVRQAPGKGLEWVSSISGSGGSTLYADSVKGRFTISRDNSKNTLYLQMNSLRAEDTAVYYCAKLTGTSFDYWGQGTLVTVSSASTKGPSVFPLAPSSKSTSGGTAALGCLVKDYFPEPVTVSWNSGALTSGVHTFPAVLQSSGLYSLSSVVTVPSSSLGTQTYICNVNHKPSNTKVDKKVEPKSCDKTHTCPPCPAPELLGGPSVFLFPPKPKDTLMISRTPEVTCVVVDVSHEDPEVKFNWYVDGVEVHNAKTKPREEQYNSTYRVVSVLTVLHQDWLNGKEYKCKVSNKALPAPIEKTISKAKGQPREPQVYTLPPSRDELTKNQVSLTCLVKGFYPSDIAVEWESNGQPENNYKTTPPVLDSDGSFFLYSKLTVDKSRWQQGNVFSCSVMHEALHNHYTQKSLSLSPG

SEQ ID NO: 60 - protein, 215 aa, unidentified
QSVLTQPPSASGTPGQRVTISCSGSSSNIGSNPVNWYQQLPGTAPKLLIYSNNQRPSGVPDRFSGSKSGTSASLAITGLQSEDEADYYCQSFDSSLKKVFGGGTKLTVLGQPKAAPSVTLFPPSSEELQANKATLVCLISDFYPGAVTVAWKADSSPVKAGVETTTPSKQSNNKYAASSYLSLTPEQWKSHRSYSCQVTHEGSTVEKTVAPTECS

SEQ ID NO: 61 - protein, 446 aa, unidentified
EVQLLESGGGLVQPGGSLRLSCAASGFTFSSYAMSWVRQAPGKGLEWVSSISGSGGSTLYADSVKGRFTISRDNSKNTLYLQMNSLRAEDTAVYYCAKLTGTSFDYWGQGTLVTVSSASTKGPSVFPLAPSSKSTSGGTAALGCLVKDYFPEPVTVSWNSGALTSGVHTFPAVLQSSGLYSLSSVVTVPSSSLGTQTYICNVNHKPSNTKVDKKVEPKSCDKTHTCPPCPAPELLGGPSVFLFPPKPKDTLMISRTPEVTCVVVDVSHEDPEVKFNWYVDGVEVHNAKTKPREEQYASTYRVVSVLTVLHQDWLNGKEYKCKVSNKALPAPIEKTISKAKGQPREPQVYTLPPSRDELTKNQVSLTCLVKGFYPSDIAVEWESNGQPENNYKTTPPVLDSDGSFFLYSKLTVDKSRWQQGNVFSCSVMHEALHNHYTQKSLSLSPG

SEQ ID NO: 62 - protein, 446 aa, unidentified
EVQLLESGGGLVQPGGSLRLSCAASGFTFSSYAMSWVRQAPGKGLEWVSSISGSGGSTLYADSVKGRFTISRDNSKNTLYLQMNSLRAEDTAVYYCAKLTGTSFDYWGQGTLVTVSSASTKGPSVFPLAPSSKSTSGGTAALGCLVKDYFPEPVTVSWNSGALTSGVHTFPAVLQSSGLYSLSSVVTVPSSSLGTQTYICNVNHKPSNTKVDKKVEPKSCDKTHTCPPCPAPELLGGPSVFLFPPKPKDTLMISRTPEVTCVVVDVSHEDPEVKFNWYVDGVEVHNAKTKPREEQYQSTYRVVSVLTVLHQDWLNGKEYKCKVSNKALPAPIEKTISKAKGQPREPQVYTLPPSRDELTKNQVSLTCLVKGFYPSDIAVEWESNGQPENNYKTTPPVLDSDGSFFLYSKLTVDKSRWQQGNVFSCSVMHEALHNHYTQKSLSLSPG

SEQ ID NO: 63 - protein, 118 aa, unidentified
EVQLLESGGGLVQPGGSLRLSCAASGFTFSSYGMHWVRQAPGKGLEWVSAISGSGGSTYYADSVKGRFTISRDNSKNTLYLQMNSLRAEDTAVYYCARGYYYYGMDVWGQGTLVTVSS

SEQ ID NO: 64 - protein, 5 aa, unidentified
SYGMH

SEQ ID NO: 65 - protein, 447 aa, unidentified
EVQLLESGGGLVQPGGSLRLSCAASGFTFSSYGMHWVRQAPGKGLEWVSAISGSGGSTYYADSVKGRFTISRDNSKNTLYLQMNSLRAEDTAVYYCARGYYYYGMDVWGQGTLVTVSSASTKGPSVFPLAPSSKSTSGGTAALGCLVKDYFPEPVTVSWNSGALTSGVHTFPAVLQSSGLYSLSSVVTVPSSSLGTQTYICNVNHKPSNTKVDKKVEPKSCDKTHTCPPCPAPELLGGPSVFLFPPKPKDTLMISRTPEVTCVVVDVSHEDPEVKFNWYVDGVEVHNAKTKPREEQYNSTYRVVSVLTVLHQDWLNGKEYKCKVSNKALPAPIEKTISKAKGQPREPQVYTLPPSRDELTKNQVSLTCLVKGFYPSDIAVEWESNGQPENNYKTTPPVLDSDGSFFLYSKLTVDKSRWQQGNVFSCSVMHEALHNHYTQKSLSLSPG

SEQ ID NO: 66 - protein, 447 aa, unidentified
EVQLLESGGGLVQPGGSLRLSCAASGFTFSSYGMHWVRQAPGKGLEWVSAISGSGGSTYYADSVKGRFTISRDNSKNTLYLQMNSLRAEDTAVYYCARGYYYYGMDVWGQGTLVTVSSASTKGPSVFPLAPSSKSTSGGTAALGCLVKDYFPEPVTVSWNSGALTSGVHTFPAVLQSSGLYSLSSVVTVPSSSLGTQTYICNVNHKPSNTKVDKKVEPKSCDKTHTCPPCPAPELLGGPSVFLFPPKPKDTLMISRTPEVTCVVVDVSHEDPEVKFNWYVDGVEVHNAKTKPREEQYASTYRVVSVLTVLHQDWLNGKEYKCKVSNKALPAPIEKTISKAKGQPREPQVYTLPPSRDELTKNQVSLTCLVKGFYPSDIAVEWESNGQPENNYKTTPPVLDSDGSFFLYSKLTVDKSRWQQGNVFSCSVMHEALHNHYTQKSLSLSPG

SEQ ID NO: 67 - protein, 447 aa, unidentified
EVQLLESGGGLVQPGGSLRLSCAASGFTFSSYGMHWVRQAPGKGLEWVSAISGSGGSTYYADSVKGRFTISRDNSKNTLYLQMNSLRAEDTAVYYCARGYYYYGMDVWGQGTLVTVSSASTKGPSVFPLAPSSKSTSGGTAALGCLVKDYFPEPVTVSWNSGALTSGVHTFPAVLQSSGLYSLSSVVTVPSSSLGTQTYICNVNHKPSNTKVDKKVEPKSCDKTHTCPPCPAPELLGGPSVFLFPPKPKDTLMISRTPEVTCVVVDVSHEDPEVKFNWYVDGVEVHNAKTKPREEQYQSTYRVVSVLTVLHQDWLNGKEYKCKVSNKALPAPIEKTISKAKGQPREPQVYTLPPSRDELTKNQVSLTCLVKGFYPSDIAVEWESNGQPENNYKTTPPVLDSDGSFFLYSKLTVDKSRWQQGNVFSCSVMHEALHNHYTQKSLSLSPG

SEQ ID NO: 68 - protein, 110 aa, unidentified
QSVLTQPPSASGTPGQRVTISCSGGSSNIGSNPVNWYQQLPGTAPKLLIYGNNKRPSGVPDRFSGSKSGTSASLAISGLRSEDEADYYCQSYDSSLSGWVFGGGTKLTVL

SEQ ID NO: 69 - protein, 7 aa, unidentified
GNNKRPS

SEQ ID NO: 70 - protein, 216 aa, unidentified
QSVLTQPPSASGTPGQRVTISCSGGSSNIGSNPVNWYQQLPGTAPKLLIYGNNKRPSGVPDRFSGSKSGTSASLAISGLRSEDEADYYCQSYDSSLSGWVFGGGTKLTVLGQPKAAPSVTLFPPSSEELQANKATLVCLISDFYPGAVTVAWKADSSPVKAGVETTTPSKQSNNKYAASSYLSLTPEQWKSHRSYSCQVTHEGSTVEKTVAPTECS